European Patent Application EP 4 218 789 A2, published August 2, 2023. Title: Compositions for Colon Cleansing and the Treatment of Gastrointestinal Disorders. Applicant: Ironwood Pharmaceuticals, Inc. Application EP. The sequence listing filed with the application follows.

SEQUENCE LISTING (94 sequences)

SEQ ID NO: 1 - skipped

SEQ ID NO: 2 - protein, 14 aa, synthetic construct
  REGION 1..14: note = Synthetically generated peptide
  MOD_RES 1: note = allylglycine
  MOD_RES 6: note = allylglycine
  MOD_RES 14: note = AMIDATION
GCELCGNPACTGCY

SEQ ID NO: 3 - protein, 20 aa, synthetic construct
  REGION 1..20: note = Synthetically generated peptide
  MOD_RES 1: note = N-terminus capped with C12 alkyl carboxylic acid
  MOD_RES 1: note = glutamic acid wherein the side chain carboxylic acid forms the peptide linkage
  MOD_RES 2: note = lysine wherein the side chain amine forms the peptide linkage
  MOD_RES 20: note = AMIDATION
EKNSSYCCELCCNPACTGCY

SEQ ID NO: 4 - protein, 20 aa, synthetic construct
  REGION 1..20: note = Synthetically generated peptide
  MOD_RES 1: note = N-terminus capped with C16 alkyl carboxylic acid
  MOD_RES 1: note = glutamic acid wherein the side chain carboxylic acid forms the peptide linkage
  MOD_RES 2: note = lysine wherein the side chain amine forms the peptide linkage
  MOD_RES 20: note = AMIDATION
EKNSSYCCELCCNPACTGCY

SEQ ID NO: 5 - protein, 20 aa, synthetic construct
  REGION 1..20: note = Synthetically generated peptide
  MOD_RES 1: note = N-terminus capped with C12 alkyl carboxylic acid
  MOD_RES 1: note = glutamic acid wherein the side chain carboxylic acid forms the peptide linkage
  MOD_RES 2: note = lysine wherein the side chain amine forms the peptide linkage
EKNSSYCCELCCNPACTGCY

SEQ ID NO: 6 - protein, 20 aa, synthetic construct
  REGION 1..20: note = Synthetically generated peptide
  MOD_RES 1: note = N-terminus capped with C14 alkyl carboxylic acid
  MOD_RES 1: note = glutamic acid wherein the side chain carboxylic acid forms the peptide linkage
  MOD_RES 2: note = lysine wherein the side chain amine forms the peptide linkage
EKNSSYCCELCCNPACTGCY

SEQ ID NO: 7 - protein, 20 aa, synthetic construct
  REGION 1..20: note = Synthetically generated peptide
  MOD_RES 1: note = N-terminus capped with C16 alkyl carboxylic acid
  MOD_RES 1: note = glutamic acid wherein the side chain carboxylic acid forms the peptide linkage
  MOD_RES 2: note = lysine wherein the side chain amine forms the peptide linkage
EKNSSYCCELCCNPACTGCY

SEQ ID NO: 8 - protein, 14 aa, synthetic construct
  REGION 1..14: note = Synthetically generated peptide
  MOD_RES 2: note = allylglycine
  MOD_RES 10: note = allylglycine
  MOD_RES 14: note = AMIDATION
CGELCCNPAGTGCY

SEQ ID NO: 9 - protein, 16 aa, synthetic construct
  REGION 1..16: note = Synthetically generated peptide
  MOD_RES 4: note = allylglycine
  MOD_RES 12: note = allylglycine
  MOD_RES 16: note = AMIDATION
NDDGELCVNVAGTGCL

SEQ ID NO: 10 - protein, 16 aa, synthetic construct
  REGION 1..16: note = Synthetically generated peptide
  MOD_RES 7: note = allylglycine
  MOD_RES 15: note = allylglycine
  MOD_RES 16: note = AMIDATION
NDDCELGVNVACTGGL

SEQ ID NO: 11 - protein, 20 aa, synthetic construct
  REGION 1..20: note = Synthetically generated peptide
  MOD_RES 1: note = N-terminus capped with C18 alkyl carboxylic acid
  MOD_RES 1: note = glutamic acid wherein the side chain carboxylic acid forms the peptide linkage
  MOD_RES 2: note = lysine wherein the side chain amine forms the peptide linkage
EKNSSYCCELCCNPACTGCY

SEQ ID NO: 12 - protein, 13 aa, synthetic construct
  REGION 1..13: note = Synthetically generated peptide
  MOD_RES 1: note = allylglycine
  MOD_RES 6: note = allylglycine
  MOD_RES 13: note = AMIDATION
GCELCGNPACTGC

SEQ ID NO: 13 - protein, 13 aa, synthetic construct
  REGION 1..13: note = Synthetically generated peptide
  MOD_RES 1: note = allylglycine
  MOD_RES 6: note = allylglycine
  MOD_RES 13: note = AMIDATION
GCELCGNPACAGC

SEQ ID NO: 14 - protein, 14 aa, synthetic construct
  REGION 1..14: note = Synthetically generated peptide
  MOD_RES 1: note = allylglycine
  MOD_RES 6: note = allylglycine
  MOD_RES 14: note = AMIDATION
GCEFCGNPACTGCY

SEQ ID NO: 15 - protein, 13 aa, synthetic construct
  REGION 1..13: note = Synthetically generated peptide
  MOD_RES 1: note = allylglycine
  MOD_RES 4: note = 4-fluorophenylalanine
  MOD_RES 6: note = allylglycine
  MOD_RES 13: note = AMIDATION
GCEFCGNPACTGC

SEQ ID NO: 16 - protein, 14 aa, synthetic construct
  REGION 1..14: note = Synthetically generated peptide
  MOD_RES 1: note = allylglycine
  MOD_RES 4: note = 4-fluorophenylalanine
  MOD_RES 6: note = allylglycine
  MOD_RES 14: note = AMIDATION
GCEFCGNPACTGCY

SEQ ID NO: 17 - protein, 14 aa, synthetic construct
  REGION 1..14: note = Synthetically generated peptide
  MOD_RES 1: note = allylglycine
  MOD_RES 4: note = 4-fluorophenylalanine
  MOD_RES 6: note = allylglycine
  MOD_RES 14: note = 4-fluorophenylalanine
  MOD_RES 14: note = AMIDATION
GCEFCGNPACTGCF

SEQ ID NO: 18 - protein, 14 aa, synthetic construct
  REGION 1..14: note = Synthetically generated peptide
  MOD_RES 5: note = allylglycine
  MOD_RES 13: note = allylglycine
  MOD_RES 14: note = AMIDATION
CCELGCNPACTGGY

SEQ ID NO: 19 - protein, 13 aa, synthetic construct
  REGION 1..13: note = Synthetically generated peptide
  MOD_RES 1: note = allylglycine
  MOD_RES 6: note = allylglycine
  MOD_RES 13: note = AMIDATION
GCEFCGNPACTGC

SEQ ID NO: 20 - protein, 14 aa, synthetic construct
  REGION 1..14: note = Synthetically generated peptide
  MOD_RES 1: note = allylglycine
  MOD_RES 6: note = allylglycine
  MOD_RES 14: note = 4-fluorophenylalanine
  MOD_RES 14: note = AMIDATION
GCEFCGNPACTGCF

SEQ ID NO: 21 - protein, 14 aa, synthetic construct
  REGION 1..14: note = Synthetically generated peptide
  MOD_RES 4: note = 4-fluorophenylalanine
  MOD_RES 14: note = AMIDATION
CCEFCCNPACTGCY

SEQ ID NO: 22 - protein, 14 aa, synthetic construct
  REGION 1..14: note = Synthetically generated peptide
  MOD_RES 4: note = 4-fluorophenylalanine
  MOD_RES 14: note = 4-fluorophenylalanine
  MOD_RES 14: note = AMIDATION
CCEFCCNPACTGCF

SEQ ID NO: 23 - protein, 14 aa, synthetic construct
  REGION 1..14: note = Synthetically generated peptide
  MOD_RES 1: note = allylglycine
  MOD_RES 6: note = allylglycine
  MOD_RES 14: note = 4-fluorophenylalanine
  MOD_RES 14: note = AMIDATION
GCELCGNPACTGCF

SEQ ID NO: 24 - protein, 15 aa, synthetic construct
  REGION 1..15: note = Synthetically generated peptide
  MOD_RES 1: note = 4-fluorophenylalanine
  MOD_RES 2: note = allylglycine
  MOD_RES 7: note = allylglycine
  MOD_RES 15: note = 4-fluorophenylalanine
  MOD_RES 15: note = AMIDATION
FGCELCGNPACTGCF

SEQ ID NO: 25 - protein, 14 aa, synthetic construct
  REGION 1..14: note = Synthetically generated peptide
  MOD_RES 1: note = allylglycine
  MOD_RES 6: note = allylglycine
  MOD_RES 14: note = AMIDATION
GCELCGNPACAGCY

SEQ ID NO: 26 - protein, 14 aa, synthetic construct
  REGION 1..14: note = Synthetically generated peptide
  MOD_RES 1: note = allylglycine
  MOD_RES 6: note = allylglycine
  MOD_RES 14: note = AMIDATION
GCELCGNPACYGCY

SEQ ID NO: 27 - protein, 14 aa, synthetic construct
  REGION 1..14: note = Synthetically generated peptide
  MOD_RES 1: note = allylglycine
  MOD_RES 6: note = allylglycine
  MOD_RES 14: note = AMIDATION
GCELCGNPACFGCY

SEQ ID NO: 28 - protein, 14 aa, synthetic construct
  REGION 1..14: note = Synthetically generated peptide
  MOD_RES 1: note = allylglycine
  MOD_RES 6: note = allylglycine
  MOD_RES 11: note = 4-fluorophenylalanine
  MOD_RES 14: note = AMIDATION
GCELCGNPACFGCY

SEQ ID NO: 29 - protein, 14 aa, synthetic construct
  REGION 1..14: note = Synthetically generated peptide
  MOD_RES 1: note = allylglycine
  MOD_RES 6: note = allylglycine
  MOD_RES 14: note = AMIDATION
GCELCGNPACTGCL

SEQ ID NO: 30 - protein, 14 aa, synthetic construct
  REGION 1..14: note = Synthetically generated peptide
  MOD_RES 1: note = allylglycine
  MOD_RES 6: note = allylglycine
  MOD_RES 14: note = cyclohexylalanine
  MOD_RES 14: note = AMIDATION
GCELCGNPACTGCA

SEQ ID NO: 31 - protein, 14 aa, synthetic construct
  REGION 1..14: note = Synthetically generated peptide
  MOD_RES 1: note = allylglycine
  MOD_RES 4: note = cyclohexylalanine
  MOD_RES 6: note = allylglycine
  MOD_RES 14: note = AMIDATION
GCEACGNPACTGCY

SEQ ID NO: 32 - protein, 14 aa, synthetic construct
  REGION 1..14: note = Synthetically generated peptide
  MOD_RES 1: note = allylglycine
  MOD_RES 6: note = allylglycine
  MOD_RES 14: note = D-Tyr
  MOD_RES 14: note = AMIDATION
GCELCGNPACTGCY

SEQ ID NO: 33 - protein, 14 aa, synthetic construct
  REGION 1..14: note = Synthetically generated peptide
  MOD_RES 1: note = allylglycine
  VARIANT 2: note = penicillamine
  MOD_RES 6: note = allylglycine
  VARIANT 10: note = penicillamine
  MOD_RES 14: note = AMIDATION
GXELCGNPAXTGCY

SEQ ID NO: 34 - protein, 15 aa, synthetic construct
  REGION 1..15: note = Synthetically generated peptide
  MOD_RES 1: note = allylglycine
  MOD_RES 6: note = allylglycine
  MOD_RES 15: note = AMIDATION
GCELCGNPACTGCLN

SEQ ID NO: 35 - protein, 15 aa, synthetic construct
  REGION 1..15: note = Synthetically generated peptide
  MOD_RES 1: note = allylglycine
  MOD_RES 6: note = allylglycine
  MOD_RES 15: note = AMIDATION
GCELCGNPACTGCYN

SEQ ID NO: 36 - protein, 15 aa, synthetic construct
  REGION 1..15: note = Synthetically generated peptide
  MOD_RES 2: note = allylglycine
  MOD_RES 7: note = allylglycine
  MOD_RES 15: note = AMIDATION
DGCELCGNPACTGCY

SEQ ID NO: 37 - protein, 16 aa, synthetic construct
  REGION 1..16: note = Synthetically generated peptide
  MOD_RES 3: note = allylglycine
  MOD_RES 8: note = allylglycine
  MOD_RES 16: note = AMIDATION
IDGCELCGNPACTGCY

SEQ ID NO: 38 - protein, 14 aa, synthetic construct
  REGION 1..14: note = Synthetically generated peptide
  MOD_RES 1: note = allylglycine
  MOD_RES 6: note = allylglycine
  MOD_RES 8: note = hydroxyproline
  MOD_RES 14: note = AMIDATION
GCELCGNPACTGCY

SEQ ID NO: 39 - protein, 13 aa, synthetic construct
  REGION 1..13: note = Synthetically generated peptide
  MOD_RES 1: note = allylglycine
  MOD_RES 6: note = allylglycine
  MOD_RES 8: note = hydroxyproline
  MOD_RES 13: note = AMIDATION
GCELCGNPACTGC

SEQ ID NO: 40 - protein, 14 aa, synthetic construct
  REGION 1..14: note = Synthetically generated peptide
  MOD_RES 1: note = allylglycine
  VARIANT 5: note = penicillamine
  MOD_RES 6: note = allylglycine
  VARIANT 13: note = penicillamine
  MOD_RES 14: note = AMIDATION
GCELXGNPACTGXY

SEQ ID NO: 41 - protein, 14 aa, synthetic construct
  REGION 1..14: note = Synthetically generated peptide
  MOD_RES 1: note = allylglycine
  VARIANT 5: note = penicillamine
  MOD_RES 6: note = allylglycine
  VARIANT 13: note = penicillamine
  MOD_RES 14: note = AMIDATION
GCELXGNPACTGXY

SEQ ID NO: 42 - protein, 14 aa, synthetic construct
  REGION 1..14: note = Synthetically generated peptide
  MOD_RES 1: note = allylglycine
  MOD_RES 6: note = allylglycine
  MOD_RES 14: note = N-methyl tyrosine
  MOD_RES 14: note = AMIDATION
GCELCGNPACYGCY

SEQ ID NO: 43 - protein, 13 aa, synthetic construct
  REGION 1..13: note = Synthetically generated peptide
  MOD_RES 1: note = allylglycine
  MOD_RES 6: note = allylglycine
GCELCGNPACYGC

SEQ ID NO: 44 - protein, 14 aa, synthetic construct
  REGION 1..14: note = Synthetically generated peptide
  MOD_RES 1: note = allylglycine
  MOD_RES 6: note = allylglycine
  MOD_RES 11: note = cyclohexylalanine
  MOD_RES 14: note = AMIDATION
GCELCGNPACAGCY

SEQ ID NO: 45 - protein, 14 aa, synthetic construct
  REGION 1..14: note = Synthetically generated peptide
  MOD_RES 1: note = allylglycine
  MOD_RES 6: note = allylglycine
  MOD_RES 14: note = AMIDATION
GCELCGNLACTGCY

SEQ ID NO: 46 - protein, 14 aa, synthetic construct
  REGION 1..14: note = Synthetically generated peptide
  MOD_RES 1: note = allylglycine
  MOD_RES 6: note = allylglycine
  VARIANT 8: note = sarcosine
  MOD_RES 14: note = AMIDATION
GCELCGNXACTGCY

SEQ ID NO: 47 - protein, 14 aa, synthetic construct
  REGION 1..14: note = Synthetically generated peptide
  MOD_RES 1: note = allylglycine
  MOD_RES 6: note = allylglycine
  MOD_RES 14: note = AMIDATION
GCELCGNVACTGCY

SEQ ID NO: 48 - protein, 14 aa, synthetic construct
  REGION 1..14: note = Synthetically generated peptide
  MOD_RES 1: note = allylglycine
  MOD_RES 6: note = allylglycine
  MOD_RES 14: note = N-methyl tyrosine
  MOD_RES 14: note = AMIDATION
GCELCGNPACYGCY

SEQ ID NO: 49 - protein, 13 aa, synthetic construct
  REGION 1..13: note = Synthetically generated peptide
  MOD_RES 1: note = allylglycine
  MOD_RES 6: note = allylglycine
GCELCGLPACYGC

SEQ ID NO: 50 - protein, 13 aa, synthetic construct
  REGION 1..13: note = Synthetically generated peptide
  MOD_RES 1: note = allylglycine
  MOD_RES 6: note = allylglycine
GCDLCGNPACYGC

SEQ ID NO: 51 - protein, 13 aa, synthetic construct
  REGION 1..13: note = Synthetically generated peptide
  MOD_RES 1: note = allylglycine
  MOD_RES 6: note = allylglycine
GCSLCGNPACYGC

SEQ ID NO: 52 - protein, 13 aa, synthetic construct
  REGION 1..13: note = Synthetically generated peptide
  MOD_RES 1: note = allylglycine
  MOD_RES 6: note = allylglycine
GCTLCGNPACYGC

SEQ ID NO: 53 - protein, 14 aa, synthetic construct
  REGION 1..14: note = Synthetically generated peptide
  MOD_RES 1: note = allylglycine with a reduced dicarba bond
  MOD_RES 6: note = allylglycine with a reduced dicarba bond
  MOD_RES 14: note = AMIDATION
GCELCGNPACTGCY

SEQ ID NO: 54 - protein, 13 aa, synthetic construct
  REGION 1..13: note = Synthetically generated peptide
  MOD_RES 1: note = allylglycine
  MOD_RES 6: note = allylglycine
GCQLCGNPACYGC

SEQ ID NO: 55 - protein, 14 aa, synthetic construct
  REGION 1..14: note = Synthetically generated peptide
  MOD_RES 1: note = allylglycine
  MOD_RES 6: note = allylglycine
  MOD_RES 14: note = AMIDATION
GCELCGLPACTGCY

SEQ ID NO: 56 - protein, 13 aa, synthetic construct
  REGION 1..13: note = Synthetically generated peptide
  MOD_RES 1: note = N-terminus capped with pentenoic acid
  MOD_RES 5: note = allylglycine
  MOD_RES 13: note = AMIDATION
CELCGNPACYGCY

SEQ ID NO: 57 - protein, 13 aa, synthetic construct
  REGION 1..13: note = Synthetically generated peptide
  MOD_RES 6: note = allylglycine
  MOD_RES 13: note = allylglycine
CCELCGNPACYGG

SEQ ID NO: 58 - protein, 12 aa, synthetic construct
  REGION 1..12: note = Synthetically generated peptide
  MOD_RES 1: note = N-terminus capped with pentenoic acid
  MOD_RES 5: note = allylglycine
CELCGNPACYGC

SEQ ID NO: 59 - protein, 13 aa, synthetic construct
  REGION 1..13: note = Synthetically generated peptide
  MOD_RES 1: note = allylglycine with a reduced dicarba bond
  MOD_RES 6: note = allylglycine with a reduced dicarba bond
GCELCGNPACYGC

SEQ ID NO: 60 - protein, 14 aa, synthetic construct
  REGION 1..14: note = Synthetically generated peptide
  MOD_RES 1: note = allylglycine
  MOD_RES 6: note = allylglycine
  MOD_RES 14: note = AMIDATION
GCELCGNVACYGCY

SEQ ID NO: 61 - protein, 13 aa, synthetic construct
  REGION 1..13: note = Synthetically generated peptide
  MOD_RES 1: note = allylglycine
  MOD_RES 6: note = allylglycine
GCELCGNVACYGC

SEQ ID NO: 62 - protein, 14 aa, synthetic construct
  REGION 1..14: note = Synthetically generated peptide
  VARIANT 2: note = cystathionine
  MOD_RES 14: note = AMIDATION
CXELCCNPACYGCY

SEQ ID NO: 63 - protein, 14 aa, synthetic construct
  REGION 1..14: note = Synthetically generated peptide
  VARIANT 1: note = cystathionine
  MOD_RES 14: note = AMIDATION
XCELCCNPACYGCY

SEQ ID NO: 64 - protein, 14 aa, synthetic construct
  REGION 1..14: note = Synthetically generated peptide
  VARIANT 1: note = cystathionine
XCELCCNPACYGCY

SEQ ID NO: 65 - protein, 14 aa, synthetic construct
  REGION 1..14: note = Synthetically generated peptide
  VARIANT 2: note = cystathionine
  MOD_RES 14: note = AMIDATION
CXELCCNVACYGCY

SEQ ID NO: 66 - protein, 14 aa, synthetic construct
  REGION 1..14: note = Synthetically generated peptide
  VARIANT 2: note = cystathionine
  MOD_RES 14: note = AMIDATION
CXELCCNVACTGCY

SEQ ID NO: 67 - protein, 14 aa, synthetic construct
  REGION 1..14: note = Synthetically generated peptide
  MOD_RES 1: note = acetylated N-terminus
  MOD_RES 2: note = cystathionine
  MOD_RES 14: note = AMIDATION
CXELCCNVACTGCY

SEQ ID NO: 68 - protein, 14 aa, synthetic construct
  REGION 1..14: note = Synthetically generated peptide
  MOD_RES 1: note = acetylated N-terminus
  VARIANT 2: note = cystathionine
  MOD_RES 14: note = ACETYLATION
CXELCCNPACYGCY

SEQ ID NO: 69 - protein, 13 aa, synthetic construct
  REGION 1..13: note = Synthetically generated peptide
  MOD_RES 1: note = acetylated N-terminus
  VARIANT 2: note = cystathionine
CXELCCNVACYGC

SEQ ID NO: 70 - protein, 13 aa, synthetic construct
  REGION 1..13: note = Synthetically generated peptide
  VARIANT 2: note = cystathionine
CXELCCNVACYGC

SEQ ID NO: 71 - protein, 13 aa, synthetic construct
  REGION 1..13: note = Synthetically generated peptide
  MOD_RES 1: note = acetylated N-terminus
  VARIANT 2: note = cystathionine
CXELCCNPACYGC

SEQ ID NO: 72 - protein, 12 aa, synthetic construct
  REGION 1..12: note = Synthetically generated peptide
  VARIANT 9: note = cystathionine
CCELCNVAXYGC

SEQ ID NO: 73 - protein, 14 aa, synthetic construct
  REGION 1..14: note = Synthetically generated peptide
  VARIANT 10: note = cystathionine
  MOD_RES 14: note = AMIDATION
CCELCCNVAXYGCY

SEQ ID NO: 74 - protein, 14 aa, synthetic construct
  REGION 1..14: note = Synthetically generated peptide
  VARIANT 10: note = cystathionine
  MOD_RES 14: note = AMIDATION
CCELCCNVAXTGCY

SEQ ID NO: 75 - protein, 13 aa, synthetic construct
  REGION 1..13: note = Synthetically generated peptide
  VARIANT 6: note = cystathionine
CCELCXNVACYGC

SEQ ID NO: 76 - protein, 14 aa, synthetic construct
  REGION 1..14: note = Synthetically generated peptide
  VARIANT 6: note = cystathionine
  MOD_RES 14: note = AMIDATION
CCELCXNVACYGCY

SEQ ID NO: 77 - protein, 14 aa, synthetic construct
  REGION 1..14: note = Synthetically generated peptide
  VARIANT 6: note = cystathionine
  MOD_RES 14: note = AMIDATION
CCELCXNVACTGCY

SEQ ID NO: 78 - protein, 13 aa, synthetic construct
  REGION 1..13: note = Synthetically generated peptide
  MOD_RES 1: note = N-terminus capped with 4-Mepip (1-methyl-piperidine-4-carboxylic acid)
  VARIANT 2: note = cystathionine
CXELCCNVACYGC

SEQ ID NO: 79 - protein, 13 aa, synthetic construct
  REGION 1..13: note = Synthetically generated peptide
  VARIANT 2: note = cystathionine
CXELCCNVACTGC

SEQ ID NO: 80 - protein, 13 aa, synthetic construct
  REGION 1..13: note = Synthetically generated peptide
  VARIANT 2: note = cystathionine
  MOD_RES 13: note = AMIDATION
CXELCCNVACTGC

SEQ ID NO: 81 - protein, 13 aa, synthetic construct
  REGION 1..13: note = Synthetically generated peptide
  VARIANT 2: note = cystathionine
CXELCCNVACFGC

SEQ ID NO: 82 - protein, 14 aa, synthetic construct
  REGION 1..14: note = Synthetically generated peptide
  MOD_RES 1: note = allylglycine
  MOD_RES 2: note = allylglycine
  MOD_RES 5: note = allylglycine
  MOD_RES 6: note = allylglycine
  MOD_RES 10: note = allylglycine
  MOD_RES 13: note = allylglycine
GGELGGNPAGTGGY

SEQ ID NO: 83 - protein, 14 aa, synthetic construct
  REGION 1..14: note = Synthetically generated peptide
  VARIANT 2: note = cystathionine
  MOD_RES 14: note = AMIDATION
CXELCCNAACTGCY

SEQ ID NO: 84 - protein, 14 aa, synthetic construct
  REGION 1..14: note = Synthetically generated peptide
  VARIANT 6: note = di-aminopropionic acid
  MOD_RES 14: note = AMIDATION
DCELCXNVACTGCY

SEQ ID NO: 85 - protein, 14 aa, synthetic construct
  REGION 1..14: note = Synthetically generated peptide
  VARIANT 2: note = cystathionine
  MOD_RES 14: note = AMIDATION
CXELCCNVACSGCY

SEQ ID NO: 86 - protein, 13 aa, synthetic construct
  REGION 1..13: note = Synthetically generated peptide
  VARIANT 1: note = cystathionine
  MOD_RES 5: note = allylglycine
  MOD_RES 13: note = AMIDATION
XELCGNVACTGCY

SEQ ID NO: 87 - protein, 14 aa, synthetic construct
  REGION 1..14: note = Synthetically generated peptide
  MOD_RES 1: note = allylglycine
  MOD_RES 6: note = allylglycine
  MOD_RES 14: note = AMIDATION
GCELCGNVACTGCY

SEQ ID NO: 88 - protein, 14 aa, synthetic construct
  REGION 1..14: note = Synthetically generated peptide
  MOD_RES 1: note = allylglycine
  MOD_RES 6: note = allylglycine
  MOD_RES 14: note = AMIDATION
GCELCGNPACTGCY

SEQ ID NO: 89 - protein, 13 aa, synthetic construct
  REGION 1..13: note = Synthetically generated peptide
  VARIANT 1: note = cystathionine
XCELCCNVACTGC

SEQ ID NO: 90 - protein, 14 aa, synthetic construct
  REGION 1..14: note = Synthetically generated peptide
  VARIANT 1: note = cystathionine
  MOD_RES 14: note = AMIDATION
XCELCCNVACTGCY

SEQ ID NO: 91 - protein, 14 aa, synthetic construct
  REGION 1..14: note = Synthetically generated peptide
  VARIANT 1: note = cystathionine
  MOD_RES 14: note = AMIDATION
XCELCCNVACYGCY

SEQ ID NO: 92 - protein, 13 aa, synthetic construct
  REGION 1..13: note = Synthetically generated peptide
  SITE 10: note = misc_feature - Xaa can be any naturally occurring amino acid
  VARIANT 13: note = cystathionine
CCELCCNVAXYGC

SEQ ID NO: 93 - protein, 21 aa, synthetic construct
  REGION 1..21: note = Synthetically generated peptide
  VARIANT 1: note = Xaa1 is glutamic acid wherein the side chain carboxylic acid forms the peptide linkage or is absent
  VARIANT 2: note = Xaa1 is lysine wherein the side chain amine forms the peptide linkage or is absent
  VARIANT 3: note = Xaa3 is Asn or is absent
  VARIANT 4: note = Xaa4 is Ser or is absent
  VARIANT 5: note = Xaa5 is Ser, Asn, Ile, or is absent
  VARIANT 6: note = Xaa6 is Tyr, Asp, 4-fluorophenylalanine ((4-F)Phe), or is absent
  VARIANT 7: note = Xaa7 is Cys, cystathionine (Cth), allylglycine (Ag), allylglycine with a reduced dicarba bond (Hag), or Asp
  VARIANT 8: note = Xaa8 is Cys, cystathionine (Cth), penicillamine (Pen), or allylglycine (Ag)
  VARIANT 9: note = Xaa9 is Glu, Asp, Ser, Thr, or Gln
  VARIANT 10: note = Xaa10 is Leu, cyclohexylalanine (Cha), Phe, or 4-fluorophenylalanine ((4-F)Phe)
  VARIANT 12: note = Xaa12 is Cys, allylglycine (Ag), Hag, or Val
  VARIANT 14: note = Xaa14 is Pro, Val, sarcosine (Sar), Leu, or Hydroxyproline (OH-Pro)
  VARIANT 17: note = Xaa17 is Tyr, Thr, cyclohexylalanine (Cha), 4-fluorophenylalanine ((4-F)Phe), Phe, or Ala
  VARIANT 20: note = Xaa20 is Tyr, Leu, 4-fluorophenylalanine ((4-F)Phe), cyclohexylalanine (Cha), D-Tyr, N-Methyl Tyr (Nme-Tyr) or is absent
  VARIANT 21: note = Xaa21 is absent or Asnt
XXXXXXXXXXCXNXACXGCXX

SEQ ID NO: 94 - protein, 14 aa, synthetic construct
  REGION 1..14: note = Synthetically generated peptide
CCELCCNPACTGCY